European Patent Specification EP 3 502 248 B1, published May 29, 2024. Title: ANTIBODIES AGAINST HMGB1, AND COMPOSITION COMPRISING SAME FOR TREATING OR PREVENTING ALZHEIMER'S DISEASE. Applicant: National University Corporation Tokyo Medical and Dental University. The sequence listing filed with the application follows.

SEQUENCE LISTING (15 sequences)

SEQ ID NO: 1 - DNA, 717 bp, Mus musculus
  CDS (1)..(702): Signal peptide, Variable Region and Constant Region of Light Chain (2C8C)
atggttttcacacctcagatacttggacttatgcttttttggatttcagcctccagaggtgatattgtgctaactcagtctccagccaccctgtctgtgactccaggagatagcgtcagtctttcctgcagggccagccaaagtattagcaacaacctacactggtatcaacaaaaatcacatgagtctccaaggcttctcatcaagtatgcttcccagtccatctctgggatcccctccaggttcagtggcagtggatcagggacagatttcactctcagtatcaacagtgtggagactgaagattttggaatgtatttctgtcaacagactaacagctggccgctcacgttcggtgctgggaccaagctggagctgaaacgggctgatgctgcaccaactgtatccatcttcccaccatccagtgagcagttaacatctggaggtgcctcagtcgtgtgcttcttgaacaacttctaccccaaagacatcaatgtcaagtggaagattgatggcagtgaacgacaaaatggcgtcctgaacagttggactgatcaggacagcaaagacagcacctacagcatgagcagcaccctcacgttgaccaaggacgagtatgaacgacataacagctatacctgtgaggccactcacaagacatcaacttcacccattgtcaagagcttcaacaggaatgagtgttagttaattaagcgg

SEQ ID NO: 2 - protein, 234 aa, Mus musculus
MVFTPQILGLMLFWISASRGDIVLTQSPATLSVTPGDSVSLSCRASQSISNNLHWYQQKSHESPRLLIKYASQSISGIPSRFSGSGSGTDFTLSINSVETEDFGMYFCQQTNSWPLTFGAGTKLELKRADAAPTVSIFPPSSEQLTSGGASVVCFLNNFYPKDINVKWKIDGSERQNGVLNSWTDQDSKDSTYSMSSTLTLTKDEYERHNSYTCEATHKTSTSPIVKSFNRNEC

SEQ ID NO: 3 - protein, 107 aa, Mus musculus
  SITE (1)..(107): Variable Region of Light Chain (2C8C)
DIVLTQSPATLSVTPGDSVSLSCRASQSISNNLHWYQQKSHESPRLLIKYASQSISGIPSRFSGSGSGTDFTLSINSVETEDFGMYFCQQTNSWPLTFGAGTKLELK

SEQ ID NO: 4 - protein, 11 aa, Mus musculus
  SITE (1)..(11): CDR1 of Light Chain (2C8C)
RASQSISNNLH

SEQ ID NO: 5 - protein, 8 aa, Mus musculus
  SITE (1)..(8): CDR2 of Light Chain (2C8C)
YASQSISG

SEQ ID NO: 6 - protein, 9 aa, Mus musculus
  SITE (1)..(9): CDR3 of Light Chain (2C8C)
QQTNSWPLT

SEQ ID NO: 7 - DNA, 711 bp, Mus musculus
  CDS (1)..(711): Signal peptide, Variable Region and Constant Region of Heavy Chain (2C8C)
atgacactgactctaaccatgggatggagctggatctttctcttcctcctgtcaggaactgcaggtgtccattgccaggtccagctgcagcagtctggacctgagctggtgaagcctggagcttcagtgaagctgtcctgcaaggcttctggctacaccttcactgactatactatacactgggtgaagcagagtcctggacagggacttgagtggattggatggatttatcctggaagtggtaatactaagtacaatgacaagttcaagggcaaggccacaatgactgcagacaaatcctccagcacagcctacatgcagctcagcagcctgacctctgaggattctgcggtctatttctgtgcaagagggtttgcttactggggccaagggactctggtcactgtctctgcagccaaaacaacagccccatcggtctatccactggcccctgtgtgtggagatacaagtggctcctcggtgactctaggatgcctggtcaagggttatttccctgagccagtgaccttgacctggaactctggatccctgtccagtggtgtgcacaccttcccagctgtcctgcagtctgacctctacaccctcagcagctcagtgactgtaacctcgagcacctggcccagccagtccatcacctgcaatgtggcccacccggcaagcagcaccaaggtggacaagaaaattggatcc

SEQ ID NO: 8 - protein, 237 aa, Mus musculus
MTLTLTMGWSWIFLFLLSGTAGVHCQVQLQQSGPELVKPGASVKLSCKASGYTFTDYTIHWVKQSPGQGLEWIGWIYPGSGNTKYNDKFKGKATMTADKSSSTAYMQLSSLTSEDSAVYFCARGFAYWGQGTLVTVSAAKTTAPSVYPLAPVCGDTSGSSVTLGCLVKGYFPEPVTLTWNSGSLSSGVHTFPAVLQSDLYTLSSSVTVTSSTWPSQSITCNVAHPASSTKVDKKIGS

SEQ ID NO: 9 - protein, 113 aa, Mus musculus
  SITE (1)..(113): Variable Region of Heavy Chain (2C8C)
QVQLQQSGPELVKPGASVKLSCKASGYTFTDYTIHWVKQSPGQGLEWIGWIYPGSGNTKYNDKFKGKATMTADKSSSTAYMQLSSLTSEDSAVYFCARGFAYWGQGTLVTVSA

SEQ ID NO: 10 - protein, 5 aa, Mus musculus
  SITE (1)..(5): CDR1 of Heavy Chain (2C8C)
DYTIH

SEQ ID NO: 11 - protein, 17 aa, Mus musculus
  SITE (1)..(17): CDR2 of Heavy Chain (2C8C)
WIYPGSGNTKYNDKFKG

SEQ ID NO: 12 - protein, 4 aa, Mus musculus
  SITE (1)..(4): CDR3 of Heavy Chain (2C8C)
GFAY

SEQ ID NO: 13 - DNA, 23 bp, Artificial Sequence
  GeneRacer 5'primer
cgactggagcacgaggacactga

SEQ ID NO: 14 - DNA, 28 bp, Artificial Sequence
  mIgG2a 3'primer
ggatccaattttcttgtccaccttggtg

SEQ ID NO: 15 - DNA, 38 bp, Artificial Sequence
  mIgk 3'primer
ccgcttaattaactaacactcattcctgttgaagctct